European Patent Specification EP 3 684 816 B1, published May 29, 2024. Title: CHIMERIC POLYPEPTIDES AND USES THEREOF. Applicant: KITE PHARMA, INC. The sequence listing filed with the application follows.

SEQUENCE LISTING (32 sequences)

SEQ ID NO: 1 - protein, 18 aa, Artificial Sequence
  source: /note="Description of Artificial Sequence: Synthetic peptide"
GSTSGSGKPGSGEGSTKG

SEQ ID NO: 2 - protein, 15 aa, Artificial Sequence
  source: /note="Description of Artificial Sequence: Synthetic peptide"
GGGGSGGGGSGGGGS

SEQ ID NO: 3 - protein, 23 aa, Artificial Sequence
  source: /note="Description of Artificial Sequence: Synthetic peptide"
  VARIANT (1)..(3): /replace="Ser"
  VARIANT (11)..(13): /replace="Ser"
  VARIANT (21)..(23): /replace="Ser"
  SITE (1)..(23): /note="Variant residues given in the sequence have no preference with respect to those in the annotations for variant positions"
GGGGKPGSGEGGGGKPGSGEGGG

SEQ ID NO: 4 - protein, 6 aa, Artificial Sequence
  source: /note="Description of Artificial Sequence: Synthetic peptide"
KPGSGE

SEQ ID NO: 5 - protein, 7 aa, Artificial Sequence
  source: /note="Description of Artificial Sequence: Synthetic peptide"
GKPGSGE

SEQ ID NO: 6 - protein, 7 aa, Artificial Sequence
  source: /note="Description of Artificial Sequence: Synthetic peptide"
GKPGSGG

SEQ ID NO: 7 - protein, 15 aa, Artificial Sequence
  source: /note="Description of Artificial Sequence: Synthetic peptide"
GGGSGKPGSGEGGGS

SEQ ID NO: 8 - protein, 16 aa, Artificial Sequence
  source: /note="Description of Artificial Sequence: Synthetic peptide"
GGGSGKPGSGEGGGGS

SEQ ID NO: 9 - protein, 15 aa, Artificial Sequence
  source: /note="Description of Artificial Sequence: Synthetic peptide"
GGGGSGKPGSGGGGS

SEQ ID NO: 10 - protein, 15 aa, Artificial Sequence
  source: /note="Description of Artificial Sequence: Synthetic peptide"
GGGGSGKPGSGEGGS

SEQ ID NO: 11 - protein, 16 aa, Artificial Sequence
  source: /note="Description of Artificial Sequence: Synthetic peptide"
GGGGSGKPGSGEGGGS

SEQ ID NO: 12 - protein, 17 aa, Artificial Sequence
  source: /note="Description of Artificial Sequence: Synthetic peptide"
GGGGSGKPGSGEGGGGS

SEQ ID NO: 13 - protein, 10 aa, Artificial Sequence
  source: /note="Description of Artificial Sequence: Synthetic peptide"
GSGKPGSGEG

SEQ ID NO: 14 - protein, 8 aa, Artificial Sequence
  source: /note="Description of Artificial Sequence: Synthetic peptide"
GKPGSGEG

SEQ ID NO: 15 - protein, 8 aa, Artificial Sequence
  source: /note="Description of Artificial Sequence: Synthetic peptide"
SGKPGSGE

SEQ ID NO: 16 - protein, 5 aa, Artificial Sequence
  source: /note="Description of Artificial Sequence: Synthetic peptide"
KPGSG

SEQ ID NO: 17 - protein, 15 aa, Artificial Sequence
  source: /note="Description of Artificial Sequence: Synthetic peptide"
STSGSGKPGSGEGST

SEQ ID NO: 18 - protein, 16 aa, Artificial Sequence
  source: /note="Description of Artificial Sequence: Synthetic peptide"
GGGGSGGGGSGGGGSG

SEQ ID NO: 19 - protein, 16 aa, Artificial Sequence
  source: /note="Description of Artificial Sequence: Synthetic peptide"
GGGGGSGGGGSGGGGS

SEQ ID NO: 20 - protein, 16 aa, Artificial Sequence
  source: /note="Description of Artificial Sequence: Synthetic peptide"
GGGGSGGGGSGGGGGS

SEQ ID NO: 21 - protein, 16 aa, Artificial Sequence
  source: /note="Description of Artificial Sequence: Synthetic peptide"
GSTSGSGKPGSGEGST

SEQ ID NO: 22 - protein, 14 aa, Artificial Sequence
  source: /note="Description of Artificial Sequence: Synthetic peptide"
GSTSGSGKPGSGEG

SEQ ID NO: 23 - protein, 13 aa, Artificial Sequence
  source: /note="Description of Artificial Sequence: Synthetic peptide"
GSTSGSGKPGSGE

SEQ ID NO: 24 - protein, 12 aa, Artificial Sequence
  source: /note="Description of Artificial Sequence: Synthetic peptide"
GSTSGSGKPGSG

SEQ ID NO: 25 - protein, 10 aa, Artificial Sequence
  source: /note="Description of Artificial Sequence: Synthetic peptide"
GSTSGSGKPG

SEQ ID NO: 26 - protein, 14 aa, Artificial Sequence
  source: /note="Description of Artificial Sequence: Synthetic peptide"
GSGKPGSGEGSTKG

SEQ ID NO: 27 - protein, 13 aa, Artificial Sequence
  source: /note="Description of Artificial Sequence: Synthetic peptide"
SGKPGSGEGSTKG

SEQ ID NO: 28 - protein, 12 aa, Artificial Sequence
  source: /note="Description of Artificial Sequence: Synthetic peptide"
GKPGSGEGSTKG

SEQ ID NO: 29 - protein, 11 aa, Artificial Sequence
  source: /note="Description of Artificial Sequence: Synthetic peptide"
KPGSGEGSTKG

SEQ ID NO: 30 - protein, 10 aa, Artificial Sequence
  source: /note="Description of Artificial Sequence: Synthetic peptide"
PGSGEGSTKG

SEQ ID NO: 31 - protein, 11 aa, Artificial Sequence
  source: /note="Description of Artificial Sequence: Synthetic peptide"
GSGKPGSGEGG

SEQ ID NO: 32 - protein, 5 aa, Artificial Sequence
  source: /note="Description of Artificial Sequence: Synthetic peptide"
GGGGS